European Patent Application EP 4 331 597 A2, published March 6, 2024. Title: CAROTENOIDS FOR TREATING OR PREVENTING NAUSEA. Applicant: The General Hospital Corporation. Application WO PCT/US2019/031814, filed May 10, 2019. The sequence listing filed with the application follows.

SEQUENCE LISTING (21 sequences)

SEQ ID NO: 1 - protein, 530 aa, Arthrobacter arilaitensis
MNHQDQEVVVIGGGFSGLASAGLLAARGCKVTLIEQQEHPGGRSGRLEREGFRFDTGPSWYLMPEVFDHWFRLMGTSTAEQLDLRELPTGYRVFFQNRQAPADFGIGAAASDLFETLEPGSAPALERYLRTAKEGYELALEHFLYDDFHSLKSLLDPRILRRAPQLAKLLSTSLQSHVARRFASNEIRQVLGYPAVFLGSSPEKTPALYQLMSHLDLADGVKYPMGGFAAVADAMAQLARKHGAQIQLGATATAIETSTGKNLAVSAVRWIDANGTLHRTPATKVIGAADVRHLEGELLPESLQTHTAKSFARKDPGPSAVLLCLGIKGKLPQLEHHNLLFTEDWSENFSRIRQGRELEPETSIYVCKPSATDPGTAPEGCENLFILVPAPALPEWGIGAADGQGDAAVEAVAEAAIDQLSAWARIDDLRERIVVRQSIGPGDFAQQYGAYRGGALGLAHTLGQSAMLRPGNRSAKVEGLYYAGSTVRPGIGVPMCLISGELAAKAVLGIKDAGPMPENRSVMRAQEAGA

SEQ ID NO: 2 - protein, 621 aa, Kocuria rhizophila
MTDGNRTTRHPTRPENAHRGSPDGGAPRTVVVGGGFAGLATAGLLARDGHRVTLLEQRDTLGGRSGRWSAEGFTFDTGPSWYLMPEVIDRWFTLMGSSADEQLDLRRLDPGYRTFFEQHLDEPPTDVRAGHAEELFERLDPGSSEALRAYLGSGAEVYDLAKKHFLYTNFSRPTDLARAEVLRNLPRLGGLLSTSMQRYVAARFRDPRQRQILGYPAVFLGASPDTAPAMYHLMSHLDLTDGVQYPVGGFAALVDAMERLVRAAGVEIVTGAEVTGIEVAPAPASLRSRVGAARARRRSAGSVTGVTWRAAAPEEGVRAGQDGAAGAPGARGAVRDADGPGGVVEGPGVVAEGRGTRTDASAEARGAGTDAPAGQPGDGEERTVTADVVIGAADLHHLQTRLLPDDFRAPESRWTHRDPGPSGVLVCLGVRGKLPQLVHHNLLFTADWDDNFGRIADGTPLAEQTSIYVSMTSATDPGTAPEGDENLFILVPSPAVPEWGRGGVRTPDTDEPGSPQVERVADAAIAQLARWAEIPDLAERIVVRRTYGPGDFEAQFNAWRGSMLGPGHTLRQSALFRPGVTDPGIEGLYYAGSSVRPGIGVPMCLISSEVVRDAVRERGGR

SEQ ID NO: 3 - protein, 566 aa, Micrococcus luteus
MSARDTALGPRTVVVGGGFAGLATAGLLARDGHRVTLLERGAVLGGRAGRWSEAGFTFDTGPSWYLMPEVIDRWFRLMGTSAAERLDLRRLDPGYRVYFEGHLHEPPVDVRTGHAETLFESLEPGAGRRLRAYLDSASRIYGLAKEHFLYTDFRRPAALAHPDVLRALPALGPQLLGGLRSHVAARFQDPRLRQILGYPAVFLGTSPDRAPAMYHLMSHLDLADGVQYPLGGFAALVDAMAEVVREAGVEIRTGVEATAVEVADRPAPAGRLGRLAARLPRPGAARGDEGRRRRPGRVTGVAWRSDDGAAGRLDADVVVAAADLHHVQTRLLPPGRRVAESTWDRRDPGPSGVLVCVGVRGSLPQLAHHTLLFTADWEDNFGRIERGEDLAADTSIYVSRTSATDPGVAPEGDENLFILVPAPAEPGWGRGGIRVRDGQGWRVDRAGDAQVEAVADRALDQLARWAGIPDLAERIVVRRTYGPGDFAADVHAWRGSLLGPGHTLAQSAMFRPSVRDADVAGLMYAGSSVRPGIGVPMCLISAEVVRDELRHDARRARPAGPGGSGT

SEQ ID NO: 4 - protein, 548 aa, Corynebacterium glutamicum
MKVSTKTPRSSGTAVVIGAGVAGLATSALLARDGWQVTVLEKNTDVGGRAGSLEISGFPGFRWDTGPSWYLMPEAFDHFFALFGACTSDYLDLVELTPGYRVFSGTHDAVDVPTGREEAIALFESIEPGAGAKLGNYLDSAADAYDIAIDRFLYNNFSTLGPLLHRDVLTRAGRLFSLLTRSLQKYVNSQFSSPVLRQILTYPAVFLSSRPTTTPSMYHLMSHTDLVQGVKYPIGGFTAVVNALHQLALENGVEFQLDSEVISINTASSRGNTSATGVSLLHNRKVQNLDADLVVSAGDLHHTENNLLPRELRTYPERYWSNRNPGIGAVLILLGVKGELPQLDHHNLFFSEDWTDDFAVVFDGPQLTRPHNASNSIYVSKPSTSEDGVAPAGYENLFVLIPTKASSSIGHGDAYMQSASASVETIASHAINQIATQAGIPDLTDRIVVKRTIGPADFEHRYHSWVGSALGPAHTLRQSAFLRGRNSSRKVNNLFYSGATTVPGVGIPMCLISAENIIKRLHADTSAGPLPEPLPPKTTPSQKTSYDH

SEQ ID NO: 5 - protein, 518 aa, Microbacterium testaceum
MSAQRIVVVGGGIAGLGTAALLADRGHDVHLFEARDALGGRAGSWEKDGFRFDTGPSWYLMPEVFDHFFRLLGTSAAEQLDLVRLDPAYRVYGPPGKGEPIDIVSGREAVRALFEKHEPGSGDNIDAYLDSAKDAYELSTSKFLYDPYSSTKGLRDPALVKRLPTLIPLLTRTLWKRVTSDFKNTRLQQILAYPAVFLGGSPFEVPSLYHLMSHLDLGDGVLYPKGGMTEIITAIEKLARGRGVTIETSAPVEAIITESGTARGVRLADGRIFAADAVVSGADLHHTENELLEEKDRQYPEKWWKDKVPSPGALLLLLGVTGELPQLTHHTLLFTDDWHTNFDAIFGENKKIPDPASIYICRPSASDDSVAPEGHENLFVLVPVPADPDSGRGGVSGAGDERIEKAADRVIAQIGEWTGIPDLAERIVVRKTIAPEDFKEDLHAWHGNSLGLAHTLNQSAIFRPKNRSRKVDNLYYAGTSVLPGIGLPMCLISAELVVKRLTGDTTAGPLAEPARAAV

SEQ ID NO: 6 - protein, 529 aa, Leifsonia xyli
MTAPRAVVIGGGIAGLATAALLARDGRPVTLLEQHGTLGGRAGRWETAGFRFDTGPSWYLMPEVFDHFFRLLGTSAAEQLDLVTLDPGYRVFAEDGRRPLDIRAAGAANRALFESVESGAGAALDRYLAGARETYGLAVDRFLYSTFASIRPLLSREVLARTGRLARLLLEPLDRYAARCVRDTVLRQILGYPAVFLGTSPDRAPSLYHLMSHLDLDDGVRYPVGGFATLIDRIVAFARAAGAELVTDARVTGIRTGVGGRRASAFGVDWVDAEGRSRHKHADIVVSAVDRRHTETQLLPPALRSSDREWKRRDPGPGAVLAMLGVRGELPQLTHHNLFFTTDWEANFERVFGADRGVPDPASLYVCKPSATDPGVAPPGHENLFVLVPVPADTSIGSGGIDGGGDRLVERTADAAIAQVAAWAGIPDLADRVVVRRTVGPGDFAAAVNAWSGGALGPAHTLRQSAFLRPGNASRRVRGLFFAGATTIPGIGLPMCLISAELAVKRLRGDTSAGPLAEPLAPARVGPVP

SEQ ID NO: 7 - protein, 304 aa, Corynebacterium glutamicum
MTHQNSPLFLKSALRLYNRASFKASHKVIEEYSTSFSLSTWLLSPRIRNDIRNLYAVVRIADEIVDGTAHAAGCSTAKIEEILDAYEIAVLAAPQQRFNTDLVLQAYGETARRCDFEQEHVIAFFASMRKDLKANTHDPDSFTTYVYGSAEVIGLLCLSVFNQGRTISKKRLEIMQNGARSLGAAFQKINFLRDLAEDQQNLGRFYFPKTSQGTLTKEQKEDLIADIRQDLAIAHDAFPEIPVQARIGVISAYLLFQKLTDRIEATPTADLLRERIRVPLHIKLSTLARATMKGLSMSIYRKNS

SEQ ID NO: 8 - protein, 289 aa, Microbacterium testaceum
MSVGPTGLALYSRTADDAAAAVIHRYSTSFGLAARLLGARPRPHVRNIYALVRVADEIVDGPAHDAGLTPERERAVLNALENEVMDAIATGFSANLVVHAFARTARECGIDADLIAPFFASMRTDIDTAEHDDLSHDAYVYGSAEVVGLMCLQVFLNAGMSAPARPAADLVDGARRLGAAFQDVNFLRDLADDADRLGRDYLDGAADDDRRTAVLDRIDADLAAAASVIPHLPPDCRAAVTAAHDLFAELSRRLRLSPAGAPRVRVPDGVKATLAARALLGRPPKGPRP

SEQ ID NO: 9 - protein, 298 aa, Leifsonia xyli subsp. xyli
MTRTETAAAAGPPTDLALYTRAAHESAATIIHQYSTSFGMVTRLLAPRVRPRVEDVYALVRIADEIVDGAAAEAGLDLADQRALLDALEADTERAMRTGYSANLVVHSFAATARDSGIGVALTRPFFASMRRDLSLVDFTADELREYVYGSAEVVGLMCLAVFLTDSPVADDRRRRLEAGARRLGAAFQKINFLRDLAADYAGLGRSYFPGIDPARLTERQKLALVVDIDGDLGAAADAIAELPGNCRRAIVAAHALFSELSDRIRATPARDLIVRRVSVPMRTKLAILLRATAGILR

SEQ ID NO: 10 - protein, 314 aa, Arthrobacter arilatensis
MTREFSSTDTTGTAALEHYSRAASRSARVVLGEYSTSFSLACRLLDASSAGHIANIYALVRLADEIVDGVAFQAGLDDPAIGACLDELEAETLRAMDRGYSTNMVVHAFAITARATGIKAELTTPFFASMRADLSTGEHDARSLQEYIYGSAEVIGLMCLQVFAAMPGAPQLNRAEEQRTKLAARSLGAAFQKVNFLRDLAQDSQELGRTYFPGMDPEGFDEQGKALLVAQINQDLAAARAGLPYLAPQAARAVCLAHDLFQELNVQLEKVPAAALLRTRISVSAPRKAMIALRVLLGAGTPSHHKLRMEVSSR

SEQ ID NO: 11 - protein, 303 aa, Kocuria rhizophila
MRTPMKLPAERAHTPLRLYTGTALASSGVVIGEYSTSFSLACRTLPGPVRRDIAGIYALVRVADEIVDGTARAAGLDDRAVRRALDGYEAAVDRALETGFSTDLVVHGFADVARRHGFGRELTEPFFASMRADLEVAEHDGASLEDYIYGSAEVVGLMCLEVFTDMPGTRAQTPEQREMLRSTARRLGAAFQKVNFLRDLGADHDQLGRTYLPGADPAHLTEDRKAALLADLDADLDAAVPGILALDRRARRAVSMAHGLFTELARRIERVPARELSTRRVSVPTAVKLQIAARAIADTEVTA

SEQ ID NO: 12 - protein, 298 aa, Micrococcus luteus
MAAPTPSPAALYTRTAHTAAAQVIRRYSTSFSWACRTLPRQARQDVATIYAMVRVADEVVDGVAVAAGLDEAGVRAALDDYERACEAAMASGFATDPVLHAFADVARRHGITPELTRPFFASMRADLGIREHGAESLDAYIHGSAEVVGLMCLQVFLSLPGTRARTPGQRQELRAQASRLGAAFQKVNFLRDLAADHHELGRTYLPGAAPGVLTEARKAELVAEVRADLDAALPGIRVLDPGAGRAVALAHGLFAALVDRIEATPAAELAHRRVRVPDHQKARIAARVLARGRRGGRR

SEQ ID NO: 13 - protein, 287 aa, Corynebacterium glutamicum
MMEKIRLILLSSRPISWINTAYPFGLAYLLNAGEIDWLFWLGIVFFLIPYNIAMYGINDVFDYESDMRNPRKGGVEGAVLPKSSHSTLLWASAISTIPFLVILFIFGTWMSSLWLTLSVLAVIAYSAPKLRFKERPFIDALTSSTHFTSPALIGATITGTSPSAAMWIALGSFFLWGMASQILGAVQDVNADREANLSSIATVIGARGAIRLSVVLYLLAAVLVTTLPNPAWIIGIAILTYVFNAARFWNITDASCEQANRSWKVFLWLNYFVGAVITILLIAIHQI

SEQ ID NO: 14 - protein, 287 aa, Arthrobacter arilaitensis
MIRGIVASSRPISWVNTAYPFAAAYLLAGGGVDWKFILGTVFFLFPYNLLMYGVNDVFDYESDMRNPRKGGIEGAVLSKQSHKALLIACTVCSLPFLIVLAAGGDAASNITLAVSIFAVLAYSAPRLRFKERPGLDSLTSAVHFVSPAVYGWVLAGSAVQAEQWMVFLAFLLWGMASHALGAIQDIIPDRQGGLGSIATVLSARKTIYLVLACYLLAGGLVAVGVSGIGRWAAVLSLPYVLNVLPHLGISDASSGTVNRGWKRFLWINYLCGFLLTMLLIFSAFFTY

SEQ ID NO: 15 - protein, 298 aa, Kocuria rhizophila
MPRREVDVLTRLFWASRPLSWVNTAYPFTAAVLLTGGLPWWLVVLGTVFFLVPYNLAMYGINDVFDYESDLRNPRKGGVEGAVVDRAAQRPVLLASCLVPAPFVLVLGGYAVVTGNWVSIAVLAVSLFAVVAYSWAGLRFKERPFVDAMTSATHFVSPAVYGLTLAGATFTPGLWALLIGFFLWGMASQMFGAVQDVVPDREGGLASVATVLGARPTVWVAALLYALAGGLMVFTEWPGQLAALLAVPYLLNVLRFSGVTDTDSGRANAGWKTFLWLNYLTGFLVTMLLIWWAAMRPV

SEQ ID NO: 16 - protein, 294 aa, Micrococcus luteus
MIRTLFWVSRPVSWVNTAYPFAAAAILTGGLPAWLVVLGVVFFLVPYNLAMYGINDVFDFASDLRNPRKGGVEGSVLGDPAVRRRVLAWSVLLPVPFVAVLAGWSAVRGEWAAVLVLAVSLFAVVAYSWAGLRFKERPFLDAATSATHFVSPAVYGLALAGATPTPALAALLGAFFLWGMASQMFGAVQDVVPDREGGLASVATVLGARRTVLLAAGLYAAAGLLLLATDPPGPLAALLAVPYVVNTLRFRRITDATSGAAHRGWQLFLPLNYVTGFLVTLLLIGWALTRGAAA

SEQ ID NO: 17 - protein, 297 aa, Microbacterium testaceum
MTAPAALTPGRVLRELFVSSRPVSWINTAFPFAAAYLLTTRQIDATLIVGILFFLVPYNLAMYGVNDVFDYESDLRNPRKGGTHGAVLDKRMHPITLWASVLSCLPFVVYLVVVGSPLSWLVLALSLFFVVFYSAPPLRLKERPFADSVTSSIHFFSPAVYGLVLAGAVWTWQLVFVFVAFALWGIASHAFGAVQDVEADRAADISSIATARGARWTVRFALVAYALAGVAMLFTAWPGPLAGVLVIPYLVVCWPYRNVTDAESDRATAGWNRFLWLNQIAGFGTTMLLIWWWLLTA

SEQ ID NO: 18 - protein, 298 aa, Clavibacter michiganensis
MSDVRARPGAAEMLRTVALSSRPLSWVNTAFPFAAAYLTVTRELDLTAVLGTLYFLIPYNLAMYGINDVFDYESDMRNPRKGGVEGAVLARAMHRPVLLAVLVTNVPFLVYLVIVGSAASIAVLAVSVFAVIAYSLKGLRFKERPVLDSLTSSTHFTSPAVYGIVLAGGAFTPALWAILAAFFLWGVASHAFGAVQDIVADREGGISSIATVLGGAVTVRIAVLAYAAAGVAMLFTGLPGIIAAVLVIPYILSTAPFWSIRDEDAGAANRGWRRFLGLNFLSGFVVTMLLIAYWLTTA

SEQ ID NO: 19 - protein, 291 aa, Leifsonia xyli
MIVTAPPLFRQLFLASRPLSWINTAYPFAAAYLLTAREADIVFIVGTLFFLVPYNLTMYGVNDVFDYASDLRNPRKGGVEGALLDPGTHRRTLVAAAATSLPFLVFLALAGPPLSWAVLAGSLFFVLAYSVRGLRFKKVPFLDSATSSIHFVSPALYGLVLAGATFTPGLWLVLFAFFLWGVGSHAFGAVQDVAPDREAGIASVATVLGAARTVRFAIAAWALAALAALAIPWPGPLVAMLALPYITVAAPFWSVPDDRASAANRGWLRFLGINYACGCLLTLLLIGYALR

SEQ ID NO: 20 - protein, 340 aa, Caenorhabditis elegans
MYRFLSGIKVVEIAGLAPVPHCGMMLADFGADVTVIDKKNPAIEQRLNRGKTMKQLDLKNPEDIKKVRDLCQTSDVLLDPYRPGTLEKMGLDPSTLWNNNKGLIICKISGYGQTGRMSQETGHDINYVALSGMLPTFSGVNATRPWPPANMLADFAGGGLSAAFGILSAIYARSHNGGKGCLLDCSMTEGVAYLSSFVQHYYDQPNLFTDKYALFSGECPIYRTYKTKDDKFVAVGAVEPKFYQNLFKLLNVDGRDLFVNPGKITEDLESRFLQKTRDKWANIFKGQECCVTPVLDIHEVGSYGQHVDRNSFTKTSSNWIANPSPRVWTQDELAALSSKK

SEQ ID NO: 21 - protein, 343 aa, Caenorhabditis elegans
MSRLLSGIKVVELGGLAPVPFCGMILADFGADVTVIDKKNPTVEQRMNRGKSMKEFDLRKSEDIKKVRDLCRTSDVLLDPYRPGTLEKMGLDPLSLWNDNKGLIICRISGYGQTGRMSQEAGHDINYVAMSGMLPTFAGAEASRPWPPVNMLADFAGGGLSAAFGIVSAIHARTHNGGQGCVLDCSMTEGVAYLASFVQYYYEQSHLFTDKYAAFTGECPIYRTYKTKDGKFMAVGPLEPKFHQKMFQVLGVNGDDLFSEPERITKVLEETFLQKTRDEWSSIFEGQDCCVTPVLDIHEVGTYGQHVDRQNFTKNDKFGSTWIAKPSPRVKTPEELFAARSKL